European Patent Application EP 4 509 529 A1, published February 19, 2025. Title: Antibody for use in treating infection with Coronaviridae. Applicant: RIKEN. Application JP. The sequence listing filed with the application follows.

SEQUENCE LISTING (153 sequences)

SEQ ID NO: 1 - protein, 492 aa, Mesocricetus auratus
MALNSGSPPGIGPYYENHGFQSEHIYPPRPPVAPDVYNPYPPQNYPPPVPQYFPRVTTQASTTVTHTQPHSSGKLCTSTSKTKKSLCFALSLGIVLVGAAVAAVLLWKFLPGCSTSEMECMSSGTCISSSLWCDGTSHCPNGEDENRCAVRLYGPSFTLQVYSSQRKAWYPVCQDDWNDSYGRAACKDMGYKNNFYYTQGIPDSSGATSFMKLNISAGNIDLYKKLYHSDSCSSRMVVSLRCIQCGVRSATRQSRIVGGSNASPGDWPWQVSLHVQGVHVCGGSIITPEWIVTAAHCVEEPLNSPRYWTAFAGILSQSLMFYGSRHQVEKVISHPNYNSETKNNDIALMKLQTPLTFNDLVKPVCLPNPGMMLDPAQECWISGWGSTYEKGKTSDMLNAAMVPLIERSKCNNKYIYNNLITPAMVCAGFLQGTVDSCQGDSGGPLVTLKNDIWWLIGDTSWGSGCAKALRPGVYGNVTVFTDWIYQQMMANS

SEQ ID NO: 2 - protein, 490 aa, Mus musculus
MALNSGSPPGIGPCYENHGYQSEHICPPRPPVAPNGYNLYPAQYYPSPVPQYAPRITTQASTSVIHTHPKSSGALCTSKSKKSLCLALALGTVLTGAAVAAVLLWRFWDSNCSTSEMECGSSGTCISSSLWCDGVAHCPNGEDENRCVRLYGQSFILQVYSSQRKAWYPVCQDDWSESYGRAACKDMGYKNNFYSSQGIPDQSGATSFMKLNVSSGNVDLYKKLYHSDSCSSRMVVSLRCIECGVRSVKRQSRIVGGLNASPGDWPWQVSLHVQGVHVCGGSIITPEWIVTAAHCVEEPLSSPRYWTAFAGILRQSLMFYGSRHQVEKVISHPNYDSKTKNNDIALMKLQTPLAFNDLVKPVCLPNPGMMLDLDQECWISGWGATYEKGKTSDVLNAAMVPLIEPSKCNSKYIYNNLITPAMICAGFLQGSVDSCQGDSGGPLVTLKNGIWWLIGDTSWGSGCAKALRPGVYGNVTVFTDWIYQQMRANS

SEQ ID NO: 3 - protein, 492 aa, Felis catus
MALNSGPPPGVGPFYENHGYQPEGLYPPRPAVVPGAYSVYPAPYYPPAVPQYAPRVLTHASTPSSHTQPKSPSGTVCTSKAKKVLCITFTLGAVLAGAVLAAVLLWKFMENKCLVSGIECGSSGTCVSPSHWCDGVLHCPSGEDENRCVRLYGPNFILQVYSSQRKSWHPVCQDDWSEGYGRAACQDMGYRNSFYSSHGVADDSGATSFMRVNTSANHMDLYKKLYHSDVCSSKTVVSLRCIECGVTAKMGRQSRIVGGSSAAPGDWPWQASLHVQGVHVCGGSIISPEWIVTAAHCVEEPLNNPRHWTAFVGILRQSFMFYGHGYRVGKVISHPNYDSKTKNNDIALMKLQTPLTFDDKVKPVCLPNPGLMLEPEQPCWISGWGATHEKGKTSDELNAVMVPLIEPWRCNSKYVYNNLVTPAMICAGYLQGTIDSCQGDSGGPLVTMKSHIWWLIGDTSWGSGCAKANRPGVYGNVTVFTDWIYRQMRANG

SEQ ID NO: 4 - protein, 492 aa, Homo sapiens
MALNSGSPPAIGPYYENHGYQPENPYPAQPTVVPTVYEVHPAQYYPSPVPQYAPRVLTQASNPVVCTQPKSPSGTVCTSKTKKALCITLTLGTFLVGAALAAGLLWKFMGSKCSNSGIECDSSGTCINPSNWCDGVSHCPGGEDENRCVRLYGPNFILQVYSSQRKSWHPVCQDDWNENYGRAACRDMGYKNNFYSSQGIVDDSGSTSFMKLNTSAGNVDIYKKLYHSDACSSKAVVSLRCIACGVNLNSSRQSRIVGGESALPGAWPWQVSLHVQNVHVCGGSIITPEWIVTAAHCVEKPLNNPWHWTAFAGILRQSFMFYGAGYQVEKVISHPNYDSKTKNNDIALMKLQKPLTFNDLVKPVCLPNPGMMLQPEQLCWISGWGATEEKGKTSEVLNAAKVLLIETQRCNSRYVYDNLITPAMICAGFLQGNVDSCQGDSGGPLVTSKNNIWWLIGDTSWGSGCAKAYRPGVYGNVMVFTDWIYRQMRADG

SEQ ID NO: 5 - protein, 492 aa, unidentified
  REGION 1..492: note = Chlorocebus sabaeus TMPRESS2
MALNSGSPPGVGPYYENHGYQPENPYPAQPTVAPNVYEVHPAQYYPSPVPQYIPSVLTHASNPAVRTQPKSPSGTVCTSKTKKALCVTMTLGAVLVGAALAAGLLWKFMGSKCSDSGIECDSSGTCISSSNWCDGVSHCPSGEDENRCVRLYGPNFILQVYSSQRKSWHPVCRDDWNENYARAACRDMGYQNRFYSSQGIADNSGATSFMKLNTSAGNVDIYKKLYHSDACSSKAVVSLRCIACGVRSNLSRQSRIVGGQNALPGAWPWQVSLHVQNIHVCGGSIITPEWIVTAAHCVEKPLNSPWQWTAFAGILTQSSMFYVKGHRVEKVISHPNYDSKTKNNDIALMKLHTPLTFNELVKPVCLPNPGMMLEPEQHCWISGWGATQEKGKTSDMLNAAMVPLIEPRRCNSKRVYDGLVTPAMICAGFLQGTVDSCQGDSGGPLVTLKNDVWWLIGDTSWGSGCAQANRPGVYGNVTVFTDWIYRQMRADD

SEQ ID NO: 6 - protein, 492 aa, Macaca fascicularis
MALNSGSPPGVGPYYENHGYQPENPYPAQPTVAPNVYEVHPAQYYPSPVPQYTPRVLTHASNPAVCRQPKSPSGTVCTSKTKKALCVTMTLGAVLVGAALAAGLLWKFMGSKCSDSGIECDSSGTCISSSNWCDGVSHCPNGEDENRCVRLYGPNFILQVYSSQRKSWHPVCRDDWNENYARAACRDMGYKNSFYSSQGIVDNSGATSFMKLNTSAGNVDIYKKLYHSDACSSKAVVSLRCIACGVRSNLNRQSRIVGGQNALLGAWPWQVSLHVQNIHVCGGSIITPEWIVTAAHCVEKPLNSPWQWTAFVGTLRQSSMFYEKGHRVEKVISHPNYDSKTKNNDIALMKLHTPLTFNEVVKPVCLPNPGMMLEPEQHCWISGWGATQEKGKTSDVLNAAMVPLIEPRRCNNKYIYDGLITPAMICAGFLRGTVDSCQGDSGGPLVTLKNDVWWLIGDTSWGSGCAQANRPGVYGNVTVFTDWIYRQMRADD

SEQ ID NO: 7 - protein, 492 aa, Macaca mulatta
MALNSGSPPGVGPYYENHGYQPENPYPAQPTVAPNVYEVHPAQYYPSPVPQYTPRVLTHASNPAVCRQPKSPSGTVCTSKTKKALCVTMTLGAVLVGAALAAGLLWKFMGSKCSDSGIECDSSGTCISSSNWCDGVSHCPNGEDENRCVRLYGPNFILQVYSSQRKSWHPVCRDDWNENYARAACRDMGYKNSFYSSQGIVDNSGATSFMKLNTSAGNVDIYKKLYHSDACSSKAVVSLRCIACGVRSNLSRQSRIVGGQNALLGAWPWQVSLHVQNIHVCGGSIITPEWIVTAAHCVEKPLNSPWQWTAFVGTLRQSSMFYEKGHRVEKVISHPNYDSKTKNNDIALMKLHTPLTFNEVVKPVCLPNPGMMLEPEQHCWISGWGATQEKGKTSDVLNAAMVPLIEPRRCNNKYVYDGLITPAMICAGFLQGTVDSCQGDSGGPLVTLKNDVWWLIGDTSWGSGCAQANRPGVYGNVTVFTDWIYRQMRADD

SEQ ID NO: 8 - protein, 492 aa, unidentified
  REGION 1..492: note = Mustela putorius furo TMPRESS2
MALNAGSPPGVGPYYENHGYQPESLYPAPPATVPSVYVAYPAAYYPPAVPQYTPRVLTQASTPAVRTQPKSPSGTACTAKAKKALCITISLGAVLAGAAVTAVLLWKFMENKCSVSGIECGSSGTCISPSHWCDGVLHCPSGEDENRCVRLYGPNFILQVYSAQRKSWHPVCQDDWSDSYGRAACQDMGYRNSFYSSQGIVDDSGASSFMKLNTSAGNTDLYKKLYHSDICASKTVVSLRCIECGVAGKTMRQSRIVGGSSASPGDWPWQVSLHVQGTHVCGGSIITPEWIVTAAHCVEEPLNNPRYWTVFAGVLRQSFMFYGHGYRVGKVISHPSYDSKTKNNDIALMKLQTPLTFSDKVKPVCLPNPGMMLEPNQSCWISGWGATHEKGKTSDELNAVMVPLIEPWRCNSKYVYNSLVTPAMICAGYLRGGTDSCQGDSGGPLVTLKSRIWWLIGDTSWGSGCAKANRPGVYGNVTVFTDWIYRQMRANS

SEQ ID NO: 9 - protein, 120 aa, synthetic construct
  REGION 1..120: note = 752_1 VH
QVQLQQSGAELARPGASVKLSCKASGYTFTSCGISWVKQRTGQGLEWIGEIYPRGGNTYYNEKFKGKATLTADKSSSTAYMELRSLTSEDSAVYFCARENGNYDPLFAYWGQGTLVTVSA

SEQ ID NO: 10 - protein, 106 aa, synthetic construct
  REGION 1..106: note = 752_1 VL
DIQMTQSPSSLSASLGGKVTITCKASQDINKYIAWYQHKPGKGPRLLIHYTSTLQPGIPSRFSGSGSGRDYSFSIYNLEPEDIATYYCLQYYNLWTFGGGTKLEIK

SEQ ID NO: 11 - protein, 5 aa, synthetic construct
  REGION 1..5: note = 752_1 HCDR1
SCGIS

SEQ ID NO: 12 - protein, 17 aa, synthetic construct
  REGION 1..17: note = EIYPRGGNTYYNEKFKG
EIYPRGGNTYYNEKFKG

SEQ ID NO: 13 - protein, 11 aa, synthetic construct
  REGION 1..11: note = 752_1 HCDR3
ENGNYDPLFAY

SEQ ID NO: 14 - protein, 11 aa, synthetic construct
  REGION 1..11: note = 752_1 LCDR1
KASQDINKYIA

SEQ ID NO: 15 - protein, 7 aa, synthetic construct
  REGION 1..7: note = 752_1 LCDR2
YTSTLQP

SEQ ID NO: 16 - protein, 8 aa, synthetic construct
  REGION 1..8: note = 752_1 LCDR3
LQYYNLWT

SEQ ID NO: 17 - protein, 121 aa, synthetic construct
  REGION 1..121: note = 1864_10 VH
QVQLQQSGPALVKPGASLKISCEASGYTFTYYSINWVKQRPGQGLEWIGWIFPGSGSTYYNEKFKGKATLTIDKSSSTAYMLLSSLTSEDSAVYFCARSDYGSAYGYFDVWGTGTTVTVSS

SEQ ID NO: 18 - protein, 111 aa, synthetic construct
  REGION 1..111: note = 1864_10 VL
DIVLTQSPASLAVSLGQRATISCRASKSVSTSGYSYMHWYQQKPGQPPKLLIYLASNLESGVPARFSGSGSGTDFTLNIHPVEEEDAATYYCQHSRDLPLTFGAGTKLELK

SEQ ID NO: 19 - protein, 5 aa, synthetic construct
  REGION 1..5: note = 1864_10 HCDR1
YYSIN

SEQ ID NO: 20 - protein, 17 aa, synthetic construct
  REGION 1..17: note = 1864_10 HCDR2
WIFPGSGSTYYNEKFKG

SEQ ID NO: 21 - protein, 12 aa, synthetic construct
  REGION 1..12: note = 1864_10 HCDR3
SDYGSAYGYFDV

SEQ ID NO: 22 - protein, 15 aa, synthetic construct
  REGION 1..15: note = 1864_10 LCDR1
RASKSVSTSGYSYMH

SEQ ID NO: 23 - protein, 7 aa, synthetic construct
  REGION 1..7: note = 1864_10 LCDR2
LASNLES

SEQ ID NO: 24 - protein, 9 aa, synthetic construct
  REGION 1..9: note = 1864_10 LCDR3
QHSRDLPLT

SEQ ID NO: 25 - protein, 121 aa, synthetic construct
  REGION 1..121: note = 2020_12 VH
QVQLQQPGAELAKPGASVKLSCKASGYTFTSYWMHWVKQRPGQGLEWIGLIPPNSGSSNYNEKFKSKATLTVDKSSRTAYMQLSSLTSEDSAVYYCARWDYGSSYGYFDVWGTGTTVTVSS

SEQ ID NO: 26 - protein, 111 aa, synthetic construct
  REGION 1..111: note = 2020_12 VL
DIVLTQSPASLAVSLGQRATISCRASESVSTSGYSYMHWYQQKPGQPPKLLIYLASNLESGVPVRFSGSGSGTDFTLNIHPVEEEDAATYYCQHSRELPPTFGAGTKLELK

SEQ ID NO: 27 - protein, 5 aa, synthetic construct
  REGION 1..5: note = 2020_12 HCDR1
SYWMH

SEQ ID NO: 28 - protein, 17 aa, synthetic construct
  REGION 1..17: note = 2020_12 HCDR2
LIPPNSGSSNYNEKFKS

SEQ ID NO: 29 - protein, 12 aa, synthetic construct
  REGION 1..12: note = 2020_12 HCDR3
WDYGSSYGYFDV

SEQ ID NO: 30 - protein, 15 aa, synthetic construct
  REGION 1..15: note = 2020_12 LCDR1
RASESVSTSGYSYMH

SEQ ID NO: 31 - protein, 7 aa, synthetic construct
  REGION 1..7: note = 2020_12 LCDR2
LASNLES

SEQ ID NO: 32 - protein, 9 aa, synthetic construct
  REGION 1..9: note = 2020_12 LCDR3
QHSRELPPT

SEQ ID NO: 33 - protein, 121 aa, synthetic construct
  REGION 1..121: note = 2228_15 VH
QVQLQQSGPELVKPGTSVKISCKASGYTFTDYYINWVKQRPGQGLEWIGWIFPGSGSSYYNAIFKGKATLTVDTSSNTAHMSLSSLTSDDSAVYFCARGDFGNFGGFFTYWGQGTLVTVSA

SEQ ID NO: 34 - protein, 111 aa, synthetic construct
  REGION 1..111: note = 2228_15 VL
DVVVTQSPASLAVSLGQRATISCRASKSVSTSGYSFMHWYQQKPGQPPKLLIYLASNLESGVPARFSGSGSGTDFILNIHPVEEEDAATYYCQHSRELPLTFGAGTKLELK

SEQ ID NO: 35 - protein, 5 aa, synthetic construct
  REGION 1..5: note = 2228_15 HCDR1
DYYIN

SEQ ID NO: 36 - protein, 17 aa, synthetic construct
  REGION 1..17: note = 2228_15 HCDR2
WIFPGSGSSYYNAIFKG

SEQ ID NO: 37 - protein, 12 aa, synthetic construct
  REGION 1..12: note = 2228_15 HCDR3
GDFGNFGGFFTY

SEQ ID NO: 38 - protein, 15 aa, synthetic construct
  REGION 1..15: note = 2228_15 LCDR1
RASKSVSTSGYSFMH

SEQ ID NO: 39 - protein, 7 aa, synthetic construct
  REGION 1..7: note = 2228_15 LCDR2
LASNLES

SEQ ID NO: 40 - protein, 9 aa, synthetic construct
  REGION 1..9: note = 2228_15 LCDR3
QHSRELPLT

SEQ ID NO: 41 - protein, 20 aa, synthetic construct
  REGION 1..20: note = Peptide_181
AKAYRPGVYGNVMVFTDWIY

SEQ ID NO: 42 - protein, 20 aa, synthetic construct
  REGION 1..20: note = Peptide_182
AYRPGVYGNVMVFTDWIYRQ

SEQ ID NO: 43 - protein, 20 aa, synthetic construct
  REGION 1..20: note = Peptide_183
RPGVYGNVMVFTDWIYRQMR

SEQ ID NO: 44 - protein, 20 aa, synthetic construct
  REGION 1..20: note = Peptide_184
GVYGNVMVFTDWIYRQMRAD

SEQ ID NO: 45 - protein, 20 aa, synthetic construct
  REGION 1..20: note = Peptide_185
VYGNVMVFTDWIYRQMRADG

SEQ ID NO: 46 - protein, 20 aa, synthetic construct
  REGION 1..20: note = Peptide_168
DSGGPLVTSKNNIWWLIGDT

SEQ ID NO: 47 - protein, 20 aa, synthetic construct
  REGION 1..20: note = Peptide_169
GGPLVTSKNNIWWLIGDTSW

SEQ ID NO: 48 - protein, 20 aa, synthetic construct
  REGION 1..20: note = Peptide_170
PLVTSKNNIWWLIGDTSWGS

SEQ ID NO: 49 - protein, 20 aa, synthetic construct
  REGION 1..20: note = Peptide_171
VTSKNNIWWLIGDTSWGSGC

SEQ ID NO: 50 - protein, 20 aa, synthetic construct
  REGION 1..20: note = Peptide_172
SKNNIWWLIGDTSWGSGCAK

SEQ ID NO: 51 - protein, 20 aa, synthetic construct
  REGION 1..20: note = Peptide_173
NNIWWLIGDTSWGSGCAKAY

SEQ ID NO: 52 - protein, 20 aa, synthetic construct
  REGION 1..20: note = Peptide_146
VLNAAKVLLIETQRCNSRYV

SEQ ID NO: 53 - protein, 20 aa, synthetic construct
  REGION 1..20: note = Peptide_147
NAAKVLLIETQRCNSRYVYD

SEQ ID NO: 54 - protein, 20 aa, synthetic construct
  REGION 1..20: note = Peptide_148
AKVLLIETQRCNSRYVYDNL

SEQ ID NO: 55 - protein, 20 aa, synthetic construct
  REGION 1..20: note = Peptide_149
VLLIETQRCNSRYVYDNLIT

SEQ ID NO: 56 - protein, 20 aa, synthetic construct
  REGION 1..20: note = Peptide_102
WTAFAGILRQSFMFYGAGYQ

SEQ ID NO: 57 - protein, 20 aa, synthetic construct
  REGION 1..20: note = Peptide_103
AFAGILRQSFMFYGAGYQVE

SEQ ID NO: 58 - protein, 20 aa, synthetic construct
  REGION 1..20: note = Peptide_104
AGILRQSFMFYGAGYQVEKV

SEQ ID NO: 59 - protein, 20 aa, synthetic construct
  REGION 1..20: note = Peptide_105
ILRQSFMFYGAGYQVEKVIS

SEQ ID NO: 60 - protein, 20 aa, synthetic construct
  REGION 1..20: note = Peptide_106
RQSFMFYGAGYQVEKVISHP

SEQ ID NO: 61 - protein, 20 aa, synthetic construct
  REGION 1..20: note = Peptide_107
SFMFYGAGYQVEKVISHPNY

SEQ ID NO: 62 - protein, 20 aa, synthetic construct
  REGION 1..20: note = Peptide_108
MFYGAGYQVEKVISHPNYDS

SEQ ID NO: 63 - protein, 20 aa, synthetic construct
  REGION 1..20: note = Peptide_109
YGAGYQVEKVISHPNYDSKT

SEQ ID NO: 64 - protein, 20 aa, synthetic construct
  REGION 1..20: note = Peptide_093
WIVTAAHCVEKPLNNPWHWT

SEQ ID NO: 65 - protein, 20 aa, synthetic construct
  REGION 1..20: note = Peptide_094
VTAAHCVEKPLNNPWHWTAF

SEQ ID NO: 66 - protein, 20 aa, synthetic construct
  REGION 1..20: note = Peptide_095
AAHCVEKPLNNPWHWTAFAG

SEQ ID NO: 67 - protein, 20 aa, synthetic construct
  REGION 1..20: note = Peptide_096
HCVEKPLNNPWHWTAFAGIL

SEQ ID NO: 68 - protein, 20 aa, synthetic construct
  REGION 1..20: note = Peptide_097
VEKPLNNPWHWTAFAGILRQ

SEQ ID NO: 69 - protein, 20 aa, synthetic construct
  REGION 1..20: note = Peptide_098
KPLNNPWHWTAFAGILRQSF

SEQ ID NO: 70 - protein, 20 aa, synthetic construct
  REGION 1..20: note = Peptide_065
KAVVSLRCIACGVNLNSSRQ

SEQ ID NO: 71 - protein, 20 aa, synthetic construct
  REGION 1..20: note = Peptide_066
VVSLRCIACGVNLNSSRQSR

SEQ ID NO: 72 - protein, 20 aa, synthetic construct
  REGION 1..20: note = Peptide_067
SLRCIACGVNLNSSRQSRIV

SEQ ID NO: 73 - protein, 20 aa, synthetic construct
  REGION 1..20: note = Peptide_068
RCIACGVNLNSSRQSRIVGG

SEQ ID NO: 74 - protein, 20 aa, synthetic construct
  REGION 1..20: note = Peptide_069
IACGVNLNSSRQSRIVGGES

SEQ ID NO: 75 - protein, 20 aa, synthetic construct
  REGION 1..20: note = Peptide_036
WNENYGRAACRDMGYKNNFY

SEQ ID NO: 76 - protein, 20 aa, synthetic construct
  REGION 1..20: note = Peptide_023
RLYGPNFILQVYSSQRKSWH

SEQ ID NO: 77 - protein, 20 aa, synthetic construct
  REGION 1..20: note = Peptide_024
YGPNFILQVYSSQRKSWHPV

SEQ ID NO: 78 - protein, 20 aa, synthetic construct
  REGION 1..20: note = Peptide_025
PNFILQVYSSQRKSWHPVCQ

SEQ ID NO: 79 - protein, 20 aa, synthetic construct
  REGION 1..20: note = Peptide_026
FILQVYSSQRKSWHPVCQDD

SEQ ID NO: 80 - protein, 20 aa, synthetic construct
  REGION 1..20: note = Peptide_027
LQVYSSQRKSWHPVCQDDWN

SEQ ID NO: 81 - protein, 20 aa, synthetic construct
  REGION 1..20: note = Peptide_028
VYSSQRKSWHPVCQDDWNEN

SEQ ID NO: 82 - protein, 20 aa, synthetic construct
  REGION 1..20: note = Peptide_029
SSQRKSWHPVCQDDWNENYG

SEQ ID NO: 83 - protein, 20 aa, synthetic construct
  REGION 1..20: note = Peptide_030
QRKSWHPVCQDDWNENYGRA

SEQ ID NO: 84 - protein, 20 aa, synthetic construct
  REGION 1..20: note = Peptide_031
KSWHPVCQDDWNENYGRAAC

SEQ ID NO: 85 - protein, 14 aa, synthetic construct
  REGION 1..14: note = Fig6A, 1 peptide
GVYGNVMVFTDWIY

SEQ ID NO: 86 - protein, 18 aa, synthetic construct
  REGION 1..18: note = Fig6A, 2 peptide
PLVTSKNNIWWLIGDTSW

SEQ ID NO: 87 - protein, 14 aa, synthetic construct
  REGION 1..14: note = Fig6A, 3 peptide
VLLIETQRCNSRYV

SEQ ID NO: 88 - protein, 12 aa, synthetic construct
  REGION 1..12: note = Fig6A, 4 peptide
MFYGAGYQVEKV

SEQ ID NO: 89 - protein, 18 aa, synthetic construct
  REGION 1..18: note = Fig6A, 5 peptide
VTAAHCVEKPLNNPWHWT

SEQ ID NO: 90 - protein, 20 aa, synthetic construct
  REGION 1..20: note = Fig6A, 6 peptide
KPLNNPWHWTAFAGILRQSF

SEQ ID NO: 91 - protein, 14 aa, synthetic construct
  REGION 1..14: note = Fig6B, 7 peptide
IACGVNLNSSRQSR

SEQ ID NO: 92 - protein, 20 aa, synthetic construct
  REGION 1..20: note = Fig6B, 8 peptide
WNENYGRAACRDMGYKNNFY

SEQ ID NO: 93 - protein, 22 aa, synthetic construct
  REGION 1..22: note = Fig6B, 9 peptide
PNFILQVYSSQRKSWHPVCQDD

SEQ ID NO: 94 - protein, 20 aa, synthetic construct
  REGION 1..20: note = Cat TMPRSS2 176-195
WSEGYGRAACQDMGYRNSFY

SEQ ID NO: 95 - protein, 18 aa, synthetic construct
  REGION 1..18: note = Cat TMPRSS2 292-306
VTAAHCVEEPLNNPRHWT

SEQ ID NO: 96 - protein, 6 aa, synthetic construct
  REGION 1..6: note = Human TMPRSS2 316-321
RQSFMF

SEQ ID NO: 97 - protein, 6 aa, synthetic construct
  REGION 1..6: note = Hamster TMPRSS2 316-321
SQSLMF

SEQ ID NO: 98 - protein, 117 aa, synthetic construct
  REGION 1..117: note = 1831_15 VH
QVQLQQPGAELVKPGASVKLSCKASGYSFTTYWMHWVRQRPGQGLEWIGIIHPNSGTTNYNEKFKSKASLTVDKSSSTAYMQLSSLTSEDSAVYYCARLLWDYFDYWGQGTTLTVSS

SEQ ID NO: 99 - protein, 112 aa, synthetic construct
  REGION 1..112: note = 1831_15 VL
DIVMSQSPSSLAVSAGEKVTMSCKSSQSLLNSRTRKNFLAWYQQKPGQSPKLLIYWASTRESGVPDRFTGSGSGTDFTLTISSVQAEDLAVYYCKQSYNLYTFGGGTKLEIK

SEQ ID NO: 100 - protein, 8 aa, synthetic construct
  REGION 1..8: note = 1831_15 HCDR1
GYSFTTYW

SEQ ID NO: 101 - protein, 8 aa, synthetic construct
  REGION 1..8: note = 1831_15 HCDR2
IHPNSGTT

SEQ ID NO: 102 - protein, 10 aa, synthetic construct
  REGION 1..10: note = 1831_15 HCDR3
ARLLWDYFDY

SEQ ID NO: 103 - protein, 12 aa, synthetic construct
  REGION 1..12: note = 1831_15 LCDR1
QSLLNSRTRKNF

SEQ ID NO: 104 - skipped

SEQ ID NO: 105 - protein, 8 aa, synthetic construct
  REGION 1..8: note = 1831_15 LCDR3
KQSYNLYT

SEQ ID NO: 106 - protein, 118 aa, synthetic construct
  REGION 1..118: note = 2114_16 VH
EVQLQQSGPELVKPGASVKISCKASGYTFTDYYMNWVKRRHGKSLEWIGNINPNNGGTSYNQKFKGKATLTVDKSSSTAYMELRSLTSEDSVVYYCAREGDLFPFAYWGQGTLVTVSA

SEQ ID NO: 107 - protein, 109 aa, synthetic construct
  REGION 1..109: note = 2114_16 VL
QAVVTQESALTTSPGETVTLTCRSSIGTVTTSNFANWVQEKPDHLFTGLIGASNNRAPGVPARFSGSLIGDKAALTITGAQTEDEAIYFCALWFSNHWVFGGGTKLTVL

SEQ ID NO: 108 - protein, 8 aa, synthetic construct
  REGION 1..8: note = 2114_16 HCDR1
GYTFTDYY

SEQ ID NO: 109 - protein, 8 aa, synthetic construct
  REGION 1..8: note = 2114_16 HCDR2
INPNNGGT

SEQ ID NO: 110 - protein, 11 aa, synthetic construct
  REGION 1..11: note = 2114_16 HCDR3
AREGDLFPFAY

SEQ ID NO: 111 - protein, 9 aa, synthetic construct
  REGION 1..9: note = 2114_16 LCDR1
IGTVTTSNF

SEQ ID NO: 112 - skipped

SEQ ID NO: 113 - protein, 9 aa, synthetic construct
  REGION 1..9: note = 2114_16 LCDR3
ALWFSNHWV

SEQ ID NO: 114 - protein, 106 aa, synthetic construct
DIQMTQSPSSLSASVGDRVTITCKASQDINKYIAWYQQKPGKAPKLLIYYTSTLQPGVPSRFSGSGSGTDFTFTISSLQPEDIATYYCLQYYNLWTFGGGTKVEIK

SEQ ID NO: 115 - protein, 23 aa, synthetic construct
DIQMTQSPSSLSASVGDRVTITC

SEQ ID NO: 116 - protein, 15 aa, synthetic construct
WYQQKPGKAPKLLIY

SEQ ID NO: 117 - protein, 32 aa, synthetic construct
GVPSRFSGSGSGTDFTFTISSLQPEDIATYYC

SEQ ID NO: 118 - protein, 10 aa, synthetic construct
FGGGTKVEIK

SEQ ID NO: 119 - protein, 106 aa, synthetic construct
DIQMTQSPSSLSASVGDRVTITCKASQDINKYIAWYQQKPGKAPKLLIHYTSTLQPGVPSRFSGSGSGTDFTFTISSLQPEDIATYYCLQYYNLWTFGGGTKVEIK

SEQ ID NO: 120 - protein, 23 aa, synthetic construct
DIQMTQSPSSLSASVGDRVTITC

SEQ ID NO: 121 - protein, 15 aa, synthetic construct
WYQQKPGKAPKLLIH

SEQ ID NO: 122 - protein, 32 aa, synthetic construct; identical to SEQ ID NO: 117

SEQ ID NO: 123 - protein, 10 aa, synthetic construct
FGGGTKVEIK

SEQ ID NO: 124 - protein, 120 aa, synthetic construct
QVQLVQSGAEVKKPGASVKVSCKASGYTFTSCGISWVRQAPGQGLEWMGEIYPRGGNTYYNEKFKGRVTMTTDTSTSTAYMELRSLRSDDTAVYYCARENGNYDPLFAYWGQGTLVTVSS

SEQ ID NO: 125 - protein, 30 aa, synthetic construct
QVQLVQSGAEVKKPGASVKVSCKASGYTFT

SEQ ID NO: 126 - protein, 14 aa, synthetic construct
WVRQAPGQGLEWMG

SEQ ID NO: 127 - protein, 32 aa, synthetic construct
RVTMTTDTSTSTAYMELRSLRSDDTAVYYCAR

SEQ ID NO: 128 - protein, 11 aa, synthetic construct
WGQGTLVTVSS

SEQ ID NO: 129 - protein, 120 aa, synthetic construct
QVQLQQSGTGLARPGASVKLSCKASGYTFTSCGISWVTQRAGQGLEWIGEIYPRGGNTYYNEKFKGKATLTADKSSSSAYMELRGLTAEDSAVYFCARENGNYDPLFAYWGQGTTLTVSS

SEQ ID NO: 130 - protein, 30 aa, synthetic construct
QVQLQQSGTGLARPGASVKLSCKASGYTFT

SEQ ID NO: 131 - protein, 14 aa, synthetic construct
WVTQRAGQGLEWIG

SEQ ID NO: 132 - protein, 32 aa, synthetic construct
KATLTADKSSSSAYMELRGLTAEDSAVYFCAR

SEQ ID NO: 133 - protein, 11 aa, synthetic construct
WGQGTTLTVSS

SEQ ID NO: 134 - protein, 111 aa, synthetic construct
DVVMTQSPLSLPVTLGQPASISCRASKSVSTSGYSFMHWFQQRPGQSPRRLIYLASNLESGVPDRFSGSGSGTDFTLKISRVEAEDVGVYYCQHSRELPLTFGGGTKVEIK

SEQ ID NO: 135 - protein, 23 aa, synthetic construct
DVVMTQSPLSLPVTLGQPASISC

SEQ ID NO: 136 - protein, 15 aa, synthetic construct
WFQQRPGQSPRRLIY

SEQ ID NO: 137 - protein, 32 aa, synthetic construct
GVPDRFSGSGSGTDFTLKISRVEAEDVGVYYC

SEQ ID NO: 138 - protein, 10 aa, synthetic construct
FGGGTKVEIK

SEQ ID NO: 139 - protein, 111 aa, synthetic construct
DIVMTQSPDSLAVSLGERATINCRASKSVSTSGYSFMHWYQQKPGQPPKLLIYLASNLESGVPDRFSGSGSGTDFTLTIRPLQAEDVAVYYCQHSRELPLTFGQGTKLEIK

SEQ ID NO: 140 - protein, 23 aa, synthetic construct
DIVMTQSPDSLAVSLGERATINC

SEQ ID NO: 141 - protein, 15 aa, synthetic construct
WYQQKPGQPPKLLIY

SEQ ID NO: 142 - protein, 32 aa, synthetic construct
GVPDRFSGSGSGTDFTLTIRPLQAEDVAVYYC

SEQ ID NO: 143 - protein, 10 aa, synthetic construct
FGQGTKLEIK

SEQ ID NO: 144 - protein, 121 aa, synthetic construct
QVQLVQSGAEVKKPGASVKVSCKASGYTFTDYYINWVRQAPGQGLEWMGWIFPGSGSSYYNAIFKGRVTMTRDTSISTAYMELSRLRSDDTAVYYCARGDFGNFGGFFTYWGQGTLVTVSS

SEQ ID NO: 145 - protein, 30 aa, synthetic construct; identical to SEQ ID NO: 125

SEQ ID NO: 146 - protein, 14 aa, synthetic construct
WVRQAPGQGLEWMG

SEQ ID NO: 147 - protein, 32 aa, synthetic construct
RVTMTRDTSISTAYMELSRLRSDDTAVYYCAR

SEQ ID NO: 148 - protein, 11 aa, synthetic construct
WGQGTLVTVSS

SEQ ID NO: 149 - protein, 121 aa, synthetic construct
EIQLVQSGAEVKKPGSSVKVSCKASGYTFTDYYINWMRQAPGQGLEWIGWIFPGSGSSYYNAIFKGRATLTVDTSTNTAYMELSSLRSEDTAFYFCARGDFGNFGGFFTYWGQGTLVTVSS

SEQ ID NO: 150 - protein, 30 aa, synthetic construct
EIQLVQSGAEVKKPGSSVKVSCKASGYTFT

SEQ ID NO: 151 - protein, 14 aa, synthetic construct
WMRQAPGQGLEWIG

SEQ ID NO: 152 - protein, 32 aa, synthetic construct
RATLTVDTSTNTAYMELSSLRSEDTAFYFCAR

SEQ ID NO: 153 - protein, 11 aa, synthetic construct
WGQGTLVTVSS